European Patent Application EP 4 477 752 A1, published December 18, 2024. Title: Antibodies or antibody fragments thereof binding to FCRL1. Applicant: 国立研究開発法人医薬基盤・健康・栄養研究所. The sequence listing filed with the application follows.

SEQUENCE LISTING (80 sequences)

SEQ ID NO: 1 - DNA, 3069 bp, Homo sapiens
  source 1..3069: mol_type = genomic DNA
gatgagctgctgctgctcgactctgaggtgcattctttttttgatgagaggcatctctaggtaccatccctgacctggtcctcatgctgccgaggctgttgctgttgatctgtgctccactctgtgaacctgccgagctgtttttgatagccagcccctcccatcccacagaggggagcccagtgaccctgacgtgtaagatgccctttctacagagttcagatgcccagttccagttctgctttttcagagacacccgggccttgggcccaggctggagcagctcccccaagctccagatcgctgccatgtggaaagaagacacagggtcatactggtgcgaggcacagacaatggcgtccaaagtcttgaggagcaggagatcccagataaatgtgcacagggtccctgtcgctgatgtgagcttggagactcagcccccaggaggacaggtgatggagggagacaggctggtcctcatctgctcagttgctatgggcacaggagacatcaccttcctttggtacaaaggggctgtaggtttaaaccttcagtcaaagacccagcgttcactgacagcagagtatgagattccttcagtgagggagagtgatgctgagcaatattactgtgtagctgaaaatggctatggtcccagccccagtgggctggtgagcatcactgtcagaatcccggtgtctcgcccaatcctcatgctcagggctcccagggcccaggctgcagtggaggatgtgctggagcttcactgtgaggccctgagaggctctcctccgatcctgtactggttttatcacgaggatatcaccctggggagcaggtcggccccctctggaggaggagcctccttcaacctttccctgactgaagaacattctggaaactactcctgtgaggccaacaatggcctgggggcccagcgcagtgaggcggtgacactcaacttcacagtgcctactggggccagaagcaatcatcttacctcaggagtcattgaggggctgctcagcacccttggtccagccaccgtggccttattattttgctacggcctcaaaagaaaaataggaagacgttcagccagggatccactcaggagccttcccagccctctaccccaagagttcacctacctcaactcacctaccccagggcagctacagcctatatatgaaaatgtgaatgttgtaagtggggatgaggtttattcactggcgtactataaccagccggagcaggaatcagtagcagcagaaaccctggggacacatatggaggacaaggtttccttagacatctattccaggctgaggaaagcaaacattacagatgtggactatgaagatgctatgtaaggttatggaagattctgctctttgaaaaccatccatgaccccaagcctcaggcctgatatgttcttcagagatcctggggcattagctttccagtatacctcttctggatgccattctccatggcactattccttcatctactgtgaagtgaagttggcgcagccctgaagaaactacctaggagaactaatagacacaggagtgacagggactttgttatcagaaccagattcctgccggctcctttgaaaacaggtcatattgtgctcttctgtttacaagaggaaacaagatggaataaaagaaattgggatcttgggttggagggacagtgaagcttagagcacatgaactcaaggttagtgactctgcaggacttcacagagagagctgtgcccatcattcagtccaagtgctttctctgcccagacagcacagaactccagccccgctacttacatggatcatcgagtttccacctaaaatatgattctatttattttgagtcactgttaccaaattagaactaaaacaaagttacataaaaagttattgtgactccacttaattttagtgacgtatttttgtatatataggccaacctataccacatccaaaattatgtatctattacagcccctagaagctttataaatacagtgtgtcttcttttattcacaaaatttttgaaatcgtggtaatatggtttgaaacctgtatcttaattattttttttttaaattgagacagggtctcactctgtcactcaatctggaatgcagtggcacaatcttgcctcactgcaacgcctgcctctcaggctcaagcaaacctctcacctcagcctgctgagtagctgggactacaggcacatgccaccaaacttggccattttttgtcttacgtagagacaagatttcaccgttttgcccaggctggtctcaaactcctgggctcaagcaatgtattgaattttaaaataaccaggcactcactcttatgaattaataaacatttggaggtatataaagtaaaaagttaaagtctttcctgtaagttaacacaaatgttaactattgttaaaaactttacaggtagctctctagatatttttctatttttgtatgtatacttatgcatacatgtaagtatataaacatttagaagtgtacctatctaacaaactattatgaaatactttcaaatctgtaaatagatctattatactattttaaaagtctctatagtagtgtgttatatagataaatcataacttttttctttttttattgtagtaaatatgcacaacataaaattgatcattttaaccatttttaagtgtacaattcagtggcattaagtactatcataatatattttaatccttctcatcactggtggacattaaggagactctcaaaaaattcatattataaaaacaaagttcaaacaaatgtctttgtactagcatattatggcactcctgctggattatctgaaggataaatttgtaaatctagtattgctagattatgcatattaaatattcttgttaaatagtcttcaatgtctctcaggtaaggctgtatcaatttatatcttcaccaacaacgtctgggaaatcagtttgtggggtgtattacttagttttcacattgctaataaagacatatccaagactgggtaatttataaa

SEQ ID NO: 2 - DNA, 5385 bp, Macaca fascicularis
  source 1..5385: mol_type = genomic DNA
ctgcaactggtggaattgaatcaaactgtatttaaaaaggagcatctttaattttctcagccttcatagaagaggaaatggagactggtcattggagggctcttcttccttctacttccgctgaagggtaacttctgatctcaacttcctcaaacctctgatgagctgctgctgctcgactctgaggtgcattgtttttttgatgagaggcatctctaggtaccatccctgacctggtcctcatgctgccgaggctgttgctgttgatctgtgctccactctgtgaacccgccgggctgttgttgatagtcagcccctcccatcccacagaggggagcccagtgaacctgacctgtaagatgccctctctacagagttcagatgcccagttccagttctgcttcttcagagatgaccaggccttgggcccgggctggagcagctctcccaagctccagatcgccaacatgtggaaagaagactcagggtcctactggtgcgaggcacagacaatggcatccaaagtcttgaggagctggagatcccagataaatgtgcacagggtccctgttgctgatgtgagcttggagactcagcccccaggaggacaggtgatggagggagacagactggtcctcatctgctcagttgctatggggacaggagacatcaccttcctttggtacaaaggggctataggtttaaaccttcagacaaagacccagcgttcactgacagcagagtatgagattcctacagcgagggagagtgatgctgagcaatactactgtgtagctgaaaatggctatggtcccagacccagtgggctggtgagcatcactgtcagaatcccagtgtctcgtcccatcctcatggtcagggctcccagggcccaggctgtggtgggggatgtgctgaagcttcactgtgaggccctgagaggctctcatccgatcctgtactggttttatcacgaggatgtcatcttggggagcagctcagccccctctggaggaggagcctctttcaacctttccctgactgcagaacattctggaaactactcctgtgaggccaacaatggcctgggggcccagcgcagtgaggaggtgacactcaacttcacagtgcctactggggccagaagcaatcatcttacctccggagtcattgaggggctcctcggcacccttggtcctgccactgtggccttattattttgctacggcctcaaaagaaaaataggaagacgttcaaccagggatccactcaggagccttcccagccctgtaccccaagagttcccctacctcaactcacctaccccaggacagctacagcctacatatgaaaatgtgaatgttgtaagtgggcgtgatgtttattcgttggtgtactataaccagccggagcaggaatcagcagcagaaaccctggggacacatatggaggaccaggtttccttagacatctattccaggctgaggaaagcaaacattacggatgtggactatgaagacgctatgtaaggttatggaggattctgccctttgaaaaccatccatgaccccaagcctcagacctgatatgttcttcagagatcctggggcattagctttccagtatacctcttctggatgctattctccgtggcactattccttcatctactgatctactgtgaagtgaagttggcgcagccctgaagaaactacctaggagaaccaatagacacaggagtgacgggaactttgttatcagaaccagattcctgctggctcttttgagaaaggtcaacttgtgctcttctatttacaagagaaaacaggatggaataaaataaattaggatcttggggtggagggacagtgaagcttagagcacatgaactcaaggtcagtgattctgcaggacttcacagagagagctgtgaccatcatcattcagtccaagtgctttctctgcccagacagcacagaactccagcactgccacttacatgggtcatcgagtttccacctaaaatatgattctatttattttgagtcactgttaccaaattagaattaaaacaaagttacataaaaagttattgtgattacacttaattttagtcacatattctgtatatataggccaacctataccacatccaaaattatgtatctactacagcccctagaagctttatgaatacagtgtgtctttttttattcacaaaatttttgaaatcttggtaatatggtttgaagtctgtatcttattttttcttttttaaatttgagacagggtctcactctgtcacccagtttggaatgcagtggcacaatctcacctcactgcaacctctgcctctcaggctcaagcaaacctctgacctcagcctcctaagtggctgggactacaggcacatgccaccaaacctggctgattttcgtcttatgtacagaccagatgtcaccattttgcccagactggtctcaaactcctgggctcaagcaatgtattttaattttaaaacaacgagacgctcattcttatgaatgaataaacatttggaggtatataaagtaaaaagttaaagtctttcctgtaagttaacacaaatgtttactattgctaaaacctttacaggtagctctctagataattttcgatttttgtgtacatacttatacatacatgtaagtatataaacatttagaagtatacctatctaacaaaccatcatgaaatattttcaaatagatctattatactattttaaaagtctcaatagtagtgtgttatatagataaatcataacttttttcttttttattgtagcaaagatacataacataaaattgatcattttaaccatgtttaagtgtacagttcagtggcattaagtactatcataatatattttaatccttctcaccactggtggacattaaggaggttccaaaaaaattcatattataaaaacaaagttcaaacaaatgtctttgtacaagcatattatgcactcctcctggactatctgaaggataaatttgtaaatctagtattgctagattatgcatattaaatattcttgttaaatagtcttcaatgtttctaaggtaaggctgtatcaatttatacctccacccataacatctgggaaatcagtttgtggggtgtgtccgttagttctcacattgctaacaaagacatacccaagactgggcaatttataaaggaaagaggtttaattgacacacagttccaaatggctagagaggcctccggacacttataatcatggcagaagaggaagcaaacatgtccttcttcacatggcagcaggagagagaaagagtcctgtgttcagcctttgcccattttctatgtcatttgtgtttttcttacagtttttataggaactatttattaagacataatttataacagtgaaatacacagattttatgtgcatagttccatcagtttgacaaatgtatgcattcaagtaatccaaacccttatcatgatttaaagtattttcatcactctagaaagttccctcatactcatgtccagtctatttatgccactctgaaaacaactactgaacattatgcttttgaccatttctccattgtatgtgatgccaatatttttgtacaatctttcacttcactttttgtttacagtgaattttaaaatatggaaggttagtttttgcacagctgaactcaattttttaaaatcttgacttctaagtttcctatatttctgtcattttctatcagaccatgttgccatgttataaaacattctaatattttcttacaatgcctccatagttttattatatattcactcaatacattatgtgtatatgtggtatgaggtaggaatctaacttttactgtttttatctttatgtattttttttaatttaaaatgaggggtagggatttaactttttttcaaacacatataaattgttcactactgtttatttaaatagtctgttcttttcccttttattattattctattttatctcacttaaattcaacctaagcctgttttggactacaactaatactacagatcttcctaccacacttccccttgcataattcacttcaaacacattagtctcaggtttcctcaggcacatcaaatttagtcccagctcagaactctgtactttctatttccatgctttcatgttctttctcttgatatccttgctttcttattttcttcatttacattttctgttttgattttctgtttctggtccatggaaattttcattttctttttataaaactaacacagcttttttacattttatattttgcctgccagtgccatgtgcctggagctcatggagggcctcaaaggatgaaattggagtatcatgtgatcaggagtttgaacttgtttgtattgtatgatcatcccttctttaccttaatactcacattaaacattatctatggcttcttacattccacttcttcttaatcaatttctttctttaagaacttaaactttcccatcatttctgatagggtctgtgagtttatttgtccaaaaagtccaaaagcagaatttaagatcaatagcatagctttctgcacaacagttgtcatattttattctatggtcttctagcttctactactttctttgagaaatctatttaattgttgtttctttataattaatctatcttttctctccagttgcctttaagacttttatatttgatattatgcaatttcactatgatttgtctaaatgtggatttattttgctagagattcataactcaagtcgaaggtatcatgccttttttcaagtttagaaaatatccggttattatctctttattattatgctgctgcagcattatttgaattctttccctcagaaatttatgttagaagtttcctagacttcattctattctcatgactcttaattagtcttgccaaattttcatttcattatctcattgcattttaggtaatttcttaatctctatcttccagtttgctagttctttcttcaactgtttatctattttattgtttaacctatttattttctatttcaatgattacattttttgagattttattagcaaaatggttaaaaggatggtttcggaggattgtctggatttacattttgcctccattatttactagctctccagttttggttaaattaattaaccttttgtgcttcttgatgtgtaaaattgaaataacaattgtatataaataaatatagtgttgttttggtaattcagtaaaattatttgtgtaaaatgcttaagacagtgcctgaaatgacattgagtcctcaaaaaataaattattattagcattatta

SEQ ID NO: 3 - protein, 429 aa, Homo sapiens
MLPRLLLLICAPLCEPAELFLIASPSHPTEGSPVTLTCKMPFLQSSDAQFQFCFFRDTRALGPGWSSSPKLQIAAMWKEDTGSYWCEAQTMASKVLRSRRSQINVHRVPVADVSLETQPPGGQVMEGDRLVLICSVAMGTGDITFLWYKGAVGLNLQSKTQRSLTAEYEIPSVRESDAEQYYCVAENGYGPSPSGLVSITVRIPVSRPILMLRAPRAQAAVEDVLELHCEALRGSPPILYWFYHEDITLGSRSAPSGGGASFNLSLTEEHSGNYSCEANNGLGAQRSEAVTLNFTVPTGARSNHLTSGVIEGLLSTLGPATVALLFCYGLKRKIGRRSARDPLRSLPSPLPQEFTYLNSPTPGQLQPIYENVNVVSGDEVYSLAYYNQPEQESVAAETLGTHMEDKVSLDIYSRLRKANITDVDYEDAM

SEQ ID NO: 4 - protein, 437 aa, Macaca fascicularis
MLPRLLLLICAPLCEPAGLLLIVSPSHPTEGSPVNLTCKMPSLQSSDAQFQFCFFRDDQALGPGWSSSPKLQIANMWKEDSGSYWCEAQTMASKVLRSWRSQINVHRVPVADVSLETQPPGGQVMEGDRLVLICSVAMGTGDITFLWYKGAIGLNLQTKTQRSLTAEYEIPTARESDAEQYYCVAENGYGPRPSGLVSITVRIPVSRPILMVRAPRAQAVVGDVLKLHCEALRGSHPILYWFYHEDVILGSSSAPSGGGASFNLSLTAEHSGNYSCEANNGLGAQRSEEVTLNFTVPTGARSNHLTSGVIEGLLGTLGPATVALLFCYGLKRKIGRRSTRDPLRSLPSPVPQEFPYLNSPTPGQLQPTYENVNVVSGRDVYSLVYYNQPEQESAAAETLGTHMEDQFAAYQDHLCSLPVGYRHSENAGLGPRFFKRP

SEQ ID NO: 5 - protein, 116 aa, Mus musculus
EVQLQESGPSLVKPSQTLSLTCSVTGDSITSGYWTWIRKFPGNKLEYMGYISYSGSTYYNPSLKSRISITRDTSKNQYYLQLNSVTTEDTATYYCARSYYYGMDSWGQGTSVTVSS

SEQ ID NO: 6 - protein, 111 aa, Mus musculus
DIVLTQSPASLAVSLGQRATISCRASESVDSYGNSFMHWYQQKPGQPPRLLIFRASNLESGIPARFSGSGSRTDFTLTINPVEADDVATYYCQQSNEDPYTFGGGTKLEIK

SEQ ID NO: 7 - protein, 118 aa, Mus musculus
EVKLEESGGGLVQPGGSMKLSCAASGFTFGDAWMDWVRQSPEKGLEWVAEIRSKANNHATYYAESVKGRFTISRDDSKSSVYLQMNSLRVEDTGIYYCTGGNYWFVYWGQGTLVTVSA

SEQ ID NO: 8 - protein, 107 aa, Mus musculus
DIVMTQSHKFMSTSVGDRVSITCKASQDVGSTVAWYQQNPGQSPKLLIYWASTRHTGVPDRFTGSGSGTDFILTISNVQSEDLADYFCQQYSSYPFTFGSGTKLEIK

SEQ ID NO: 9 - protein, 119 aa, synthetic construct
  REGION 1..119: note = Description of the artificial sequence: 1F9 VH amino acid
QLQLQESGPGLVKASETLSLTCTVSGDSISSNTFYWGWIRQPPGKGLEWIGSIYYSGSTYYNPSLKSRVTISVDTSKNQFSLKLSSVTAADTAVYYCARHEYGDFFDYWGQGTLVTVSS

SEQ ID NO: 10 - protein, 108 aa, synthetic construct
  REGION 1..108: note = Description of the artificial sequence: 1F9 VL amino acid
EIVLTQSPGTLSLSPGERATLSCRASQSVSSNYLAWFQQRPGQAPRLFIYGVSSRATGIPDRFSGSGSGTDFTLTISRLEPEDFAVYYCQQYGGSLITFGQGTRLEIK

SEQ ID NO: 11 - protein, 119 aa, synthetic construct
  REGION 1..119: note = Description of the artificial sequence: 2A10 VH amino acid
QVQLQESGPGLVKPSQTLSLTCTVSGGSISSGGYHWSWIRQHPGKGLEWIGYIYNSGSTYYNPSLKSRVTISEDTSKNQFSLKLSSVTAADSAVYYCARLVGVTYFDCWGQGTLVTVSS

SEQ ID NO: 12 - protein, 107 aa, synthetic construct
  REGION 1..107: note = Description of the artificial sequence: 2A10 VL amino acid
DIQMTQSPSSVSTSVGDRVTITCRASQGIRSWLAWYQQKPGKAPKLLIYAASSLQSGVPSRFSGSGSGTDFTLTISSLQPEDFATYYCQQANSFPPTFGQGTKVEIK

SEQ ID NO: 13 - protein, 116 aa, synthetic construct
  REGION 1..116: note = Description of the artificial sequence: 7G8 VH amino acid
DVHLVQSGGGLVHPGGSLRLSCAGSGFTFSTYTMHWIRQAPGKDLEWVSAIGTGGGTDYADSVKGRFTISRDNAKNSLYLQMNSLRAEDMAVYYCAREVYWYFDLWGRGTLVTVSS

SEQ ID NO: 14 - protein, 107 aa, synthetic construct [sequence omitted]

SEQ ID NO: 15 - protein, 117 aa, synthetic construct
  REGION 1..117: note = Description of the artificial sequence: 2G5 VH amino acid
QVQLVESGGGVVQPGRSLRLSCAASGFTFSDYGMHWVRQAPGKGLEWVAVIWYDGNNKYYADSVKGRFTISRDNSKNTLYLQMNSLRAEDTAVYYCARDWGRAFDIWGQGTMVTVSS

SEQ ID NO: 16 - protein, 108 aa, synthetic construct
  REGION 1..108: note = Description of the artificial sequence: 2G5 VL amino acid
EIVLTQSPATLSLSPGERATLSCRASQSVSSYLAWYQQKPGQAPRLLIYDASNRATGIPARFSGSGSGTDFTLTISSLEPEDFALYYCQQLNNWPPYTFGQGTKLEIK

SEQ ID NO: 17 - protein, 116 aa, synthetic construct
  REGION 1..116: note = Description of the artificial sequence: 5A2 VH amino acid
QVQVVESGGGVVQPGRSLRLSCAASGFTFSNYGMHWVRQAPGKGLEWVAGIWYDGSNKYYADSVKGRFTISRDNSKNTLYLQMNSLRAEDTAVYYCARESPNFDYWGQGTLVTVSS

SEQ ID NO: 18 - protein, 108 aa, synthetic construct
  REGION 1..108: note = Description of the artificial sequence: 5A2 VL amino acid
EIVLTQSPATLSLSPGERATLSCRASQSVSSYLAWYQQKPGQAPRLLIYDASNRATGIPARFSGSGSGTDFTLTISSLEPEDFAVYYCQQRNNWPPWTFGQGTKVEIK

SEQ ID NO: 19 - protein, 120 aa, Mus musculus
DVLLQESGPGLVKPSQSLSLTCSVAGYSITSDYAWNWLRRFPGNRLEWMGYITYSGSTAYHPSLKGRISFTRDTSQNQVFLQLHSVTTEDSATYYCAQGGTLITTWFLRWGQGTLVTVSA

SEQ ID NO: 20 - protein, 6 aa, synthetic construct
  REGION 1..6: note = Description of the artificial sequence: DK610 HCDR1 amino acid
SDYAWN

SEQ ID NO: 21 - protein, 16 aa, synthetic construct
  REGION 1..16: note = Description of the artificial sequence: DK610 HCDR2 amino acid
YITYSGSTAYHPSLKG

SEQ ID NO: 22 - protein, 11 aa, synthetic construct
  REGION 1..11: note = Description of the artificial sequence: DK610 HCDR3 amino acid
GGTLITTWFLR

SEQ ID NO: 23 - protein, 111 aa, Mus musculus
DIVLTQSPASLAVSLGQRATISCRASKSVSTSDYNYMHWYRQKPGQPPKLFIYLASNLESGVPARFSGSGSGTDFTLNIHPVEEEDAATYYCQQSRELPSTFGGGTKLEIK

SEQ ID NO: 24 - protein, 15 aa, synthetic construct
  REGION 1..15: note = Description of the artificial sequence: DK610 LCDR1 amino acid
RASKSVSTSDYNYMH

SEQ ID NO: 25 - protein, 7 aa, synthetic construct
  REGION 1..7: note = Description of the artificial sequence: DK610 LCDR2 amino acid
LASNLES

SEQ ID NO: 26 - protein, 9 aa, synthetic construct
  REGION 1..9: note = Description of the artificial sequence: DK610 LCDR3 amino acid
QQSRELPST

SEQ ID NO: 27 - protein, 117 aa, Mus musculus
QVQLQQPGAELVKPGTSVKLSCKASGYTFTRYWMHWVKQRPGQGLEWIGRIDPNSGGSKYNEKFKSKATLTVDKTSSSAYMQLNSLTSEDSAVYYCTRVNSGAMDYWGQGTSVTVSS

SEQ ID NO: 28 - protein, 5 aa, synthetic construct
  REGION 1..5: note = Description of the artificial sequence: DK681 HCDR1 amino acid
RYWMH

SEQ ID NO: 29 - protein, 17 aa, synthetic construct
  REGION 1..17: note = Description of the artificial sequence: DK681 HCDR2 amino acid
RIDPNSGGSKYNEKFKS

SEQ ID NO: 30 - protein, 8 aa, synthetic construct
  REGION 1..8: note = Description of the artificial sequence: DK681 HCDR3 amino acid
VNSGAMDY

SEQ ID NO: 31 - protein, 112 aa, Mus musculus
DIVMSQSPSSLAVSVGEKVTMSCKSSQSLLYSSNQKNYLAWYQQKPGQSPKLLIYWASTRESGVPDRFTGSGSGTDFTLTISSVKAEDLAIYYCQQYSNYPTFGSGTKLEIK

SEQ ID NO: 32 - protein, 17 aa, synthetic construct
  REGION 1..17: note = Description of the artificial sequence: DK681 LCDR1 amino acid
KSSQSLLYSSNQKNYLA

SEQ ID NO: 33 - protein, 7 aa, synthetic construct
  REGION 1..7: note = Description of the artificial sequence: DK681 LCDR2 amino acid
WASTRES

SEQ ID NO: 34 - protein, 8 aa, synthetic construct
  REGION 1..8: note = Description of the artificial sequence: DK681 LCDR3 amino acid
QQYSNYPT

SEQ ID NO: 35 - protein, 119 aa, Mus musculus
QVQLQQSGPELVKPGASVRISCKASGYTFTSYNIHWVKQRPGQGLEWIGWIYPGDGNPKYNEKFKGKTTLTADKSSSTAYMQLSSLTSEDSAVYFCARRIHYYDYFDYWGQGTTLTVSS

SEQ ID NO: 36 - protein, 5 aa, synthetic construct
  REGION 1..5: note = Description of the artificial sequence: DK1142 HCDR1 amino acid
SYNIH

SEQ ID NO: 37 - protein, 17 aa, synthetic construct
  REGION 1..17: note = Description of the artificial sequence: DK1142 HCDR2 amino acid
WIYPGDGNPKYNEKFKG

SEQ ID NO: 38 - protein, 10 aa, synthetic construct
  REGION 1..10: note = Description of the artificial sequence: DK1142 HCDR3 amino acid
RIHYYDYFDY

SEQ ID NO: 39 - protein, 112 aa, Mus musculus
DVLMTQTPLSLPVSLGDQASISCRSSQSIVHSNGNTYLEWYLQKPGQSPKLLIYKVSNRFSGVPDRFSGSGSGTDFTLKISRVEADDLGVYYCFQGSHVPWTFGGGTKLEIK

SEQ ID NO: 40 - protein, 16 aa, synthetic construct
  REGION 1..16: note = Description of the artificial sequence: DK1142 LCDR1 amino acid
RSSQSIVHSNGNTYLE

SEQ ID NO: 41 - protein, 7 aa, synthetic construct
  REGION 1..7: note = Description of the artificial sequence: DK1142 LCDR2 amino acid
KVSNRFS

SEQ ID NO: 42 - protein, 9 aa, synthetic construct
  REGION 1..9: note = Description of the artificial sequence: DK1142 LCDR3 amino acid
FQGSHVPWT

SEQ ID NO: 43 - protein, 119 aa, Mus musculus
EVRLVESGGRLVQPKGSLRLSCAVSGFTFNTYAMYWIRQAPGKGLEWVARIRSKTNNFATYYADSVKDRFTISRDDSQSMLYLQMNNLKTEDTAMYYCVRDNSGSFDYWGQGTTLTVSS

SEQ ID NO: 44 - protein, 5 aa, synthetic construct
  REGION 1..5: note = Description of the artificial sequence: DK1141 HCDR1 amino acid
TYAMY

SEQ ID NO: 45 - protein, 19 aa, synthetic construct
  REGION 1..19: note = Description of the artificial sequence: DK1141 HCDR2 amino acid
RIRSKTNNFATYYADSVKD

SEQ ID NO: 46 - protein, 8 aa, synthetic construct
  REGION 1..8: note = Description of the artificial sequence: DK1141 HCDR3 amino acid
DNSGSFDY

SEQ ID NO: 47 - protein, 112 aa, Mus musculus
DIVMAQSPSSLAVSVGEKVTMSCKSSQSLLHSSNQKNYLAWYQQKPGQSPNLLIYWASSRESGVPDRFTGSGSGTDFTLTISSVQAEDLATYYCQQYYSYPTFGAGTKLDLK

SEQ ID NO: 48 - protein, 17 aa, synthetic construct
  REGION 1..17: note = Description of the artificial sequence: DK1141 LCDR1 amino acid
KSSQSLLHSSNQKNYLA

SEQ ID NO: 49 - protein, 7 aa, synthetic construct
  REGION 1..7: note = Description of the artificial sequence: DK1141 LCDR2 amino acid
WASSRES

SEQ ID NO: 50 - protein, 8 aa, synthetic construct
  REGION 1..8: note = Description of the artificial sequence: DK1141 LCDR3 amino acid
QQYYSYPT

SEQ ID NO: 51 - protein, 119 aa, Mus musculus
QVQLQQSGPELVKPGASVRISCKASGYTFTSYNIHWVKQRPGQGLEWIGWIYPGDGNTKYNEKFKGKTTLTADKSSSTAYMQLSSLTSEDSAVYFCARRIHYFDYFDYWGQGTTLTLSS

SEQ ID NO: 52 - protein, 5 aa, synthetic construct
  REGION 1..5: note = Description of the artificial sequence: DK1166 HCDR1 amino acid
SYNIH

SEQ ID NO: 53 - protein, 17 aa, synthetic construct
  REGION 1..17: note = Description of the artificial sequence: DK1166 HCDR2 amino acid
WIYPGDGNTKYNEKFKG

SEQ ID NO: 54 - protein, 10 aa, synthetic construct
  REGION 1..10: note = Description of the artificial sequence: DK1166 HCDR3 amino acid
RIHYFDYFDY

SEQ ID NO: 55 - protein, 112 aa, Mus musculus
DVLMTQTPLSLPVSLGDQVSISCRSGQTIVHSNGNTYLEWYLQKPGQSPKLLIYKVSNRFSGVPDRFSGSGSGTDFTLRISRVEAEDLGVYYCFQGSHVPWTFGGGTKLEIK

SEQ ID NO: 56 - protein, 16 aa, synthetic construct
  REGION 1..16: note = Description of the artificial sequence: DK1166 LCDR1 amino acid
RSGQTIVHSNGNTYLE

SEQ ID NO: 57 - protein, 7 aa, synthetic construct
  REGION 1..7: note = Description of the artificial sequence: DK1166 LCDR2 amino acid
KVSNRFS

SEQ ID NO: 58 - protein, 9 aa, synthetic construct
  REGION 1..9: note = Description of the artificial sequence: DK1166 LCDR3 amino acid
FQGSHVPWT

SEQ ID NO: 59 - protein, 117 aa, Mus musculus
QVQLQQSGTELVRPGTSVKVSCKASGYAFTNYLIEWVKQRPGQGLEWIGVINPGSGGTDYNKKFKGKAMLTADKSSNTAYMQLSSLTSDDSAVYFCARSNSYAMDYWGQGTSVTVSS

SEQ ID NO: 60 - protein, 5 aa, synthetic construct
  REGION 1..5: note = Description of the artificial sequence: DK1164 HCDR1 amino acid
NYLIE

SEQ ID NO: 61 - protein, 17 aa, synthetic construct
  REGION 1..17: note = Description of the artificial sequence: DK1164 HCDR2 amino acid
VINPGSGGTDYNKKFKG

SEQ ID NO: 62 - protein, 8 aa, synthetic construct
  REGION 1..8: note = Description of the artificial sequence: DK1164 HCDR3 amino acid
SNSYAMDY

SEQ ID NO: 63 - protein, 113 aa, Mus musculus
DIVMSQSPSSLAVSVGEKVTVSCKSSQSLLYSGNQKNNLAWYKQKPGQSPKLLIYWASTRESGVPDRFTGSGSGTDFTLTMSSVKAEDLAVYYCQQYYSYPWTFGGGTKLEIK

SEQ ID NO: 64 - protein, 17 aa, synthetic construct
  REGION 1..17: note = Description of the artificial sequence: DK1164 LCDR1 amino acid
KSSQSLLYSGNQKNNLA

SEQ ID NO: 65 - protein, 7 aa, synthetic construct
  REGION 1..7: note = Description of the artificial sequence: DK1164 LCDR2 amino acid
WASTRES

SEQ ID NO: 66 - protein, 9 aa, synthetic construct
  REGION 1..9: note = Description of the artificial sequence: DK1164 LCDR3 amino acid
QQYYSYPWT

SEQ ID NO: 67 - protein, 117 aa, synthetic construct
  REGION 1..117: note = Description of the artificial sequence: hzDK681 HV0 amino acid
QVQLVQSGAEVKKPGASVKVSCKASGYTFTRYWMHWVRQAPGQGLEWMGRIDPNSGGSKYNEKFKSRVTITADTSTSTAYMELSSLRSEDTAVYYCARVNSGAMDYWGQGTLVTVSS

SEQ ID NO: 68 - protein, 112 aa, synthetic construct
  REGION 1..112: note = Description of the artificial sequence: hzDK681 LV0, DK681 F11 VL and DK681 F14 VL amino acid
DIVMTQSPDSLAVSLGERATINCKSSQSLLYSSNQKNYLAWYQQKPGQPPKLLIYWASTRESGVPDRFSGSGSGTDFTLTISSLQAEDVAVYYCQQYSNYPTFGQGTKVEIK

SEQ ID NO: 69 - protein, 119 aa, synthetic construct
  REGION 1..119: note = Description of the artificial sequence: hzDK1142 HV0 amino acid
QVQLVQSGAEVKKPGASVKVSCKASGYTFTSYNIHWVRQAPGQGLEWMGWIYPGDGNPKYNEKFKGRVTITADTSTSTAYMELSSLRSEDTAVYYCARRIHYYDYFDYWGQGTLVTVSS

SEQ ID NO: 70 - protein, 112 aa, synthetic construct
  REGION 1..112: note = Description of the artificial sequence: hzDK1142 LV0 amino acid
DIVMTQSPLSLPVTPGEPASISCRSSQSIVHSNGNTYLEWYLQKPGQSPQLLIYKVSNRFSGVPDRFSGSGSGTDFTLKISRVEAEDVGVYYCFQGSHVPWTFGQGTKVEIK

SEQ ID NO: 71 - protein, 7 aa, synthetic construct
  REGION 1..7: note = Description of the artificial sequence: DK1142 F24 LCDR2 amino acid
KISNRFS

SEQ ID NO: 72 - protein, 117 aa, synthetic construct
  REGION 1..117: note = Description of the artificial sequence: DK681 F11 and DK681 F13 VH amino acid
QVQLVQSGAELVKPGASVKVSCKASGYTFTRYWMHWVKQAPGQGLEWIGRIDPNSGGSKYNEKFKSKATLTVDKSTSTAYMELSSLRSEDTAVYYCTRVNSGAMDYWGQGTLVTVSS

SEQ ID NO: 73 - protein, 117 aa, synthetic construct
  REGION 1..117: note = Description of the artificial sequence: DK681 F12 and DK681 F14 VH amino acid
QVQLVQSGAEVKKPGASVKVSCKASGYTFTRYWMHWVKQAPGQGLEWIGRIDPNSGGSKYNEKFKSKATITVDKSTSTAYMELSSLRSEDTAVYYCTRVNSGAMDYWGQGTLVTVSS

SEQ ID NO: 74 - protein, 112 aa, synthetic construct
  REGION 1..112: note = Description of the artificial sequence: DK681 F12 and DK681 F13 VL amino acid
DIVMTQSPDSLAVSLGERATMNCKSSQSLLYSSNQKNYLAWYQQKPGQSPKLLIYWASTRESGVPDRFSGSGSGTDFTLTISSLQAEDVAIYYCQQYSNYPTFGQGTKVEIK

SEQ ID NO: 75 - protein, 119 aa, synthetic construct
  REGION 1..119: note = Description of the artificial sequence: DK1142 F21 VH amino acid
QVQLVQSGAEVKKPGASVKVSCKASGYTFTSYNIHWVRQAPGQGLEWMGWIYPGDGNPKYNEKFKGKTTLTADKSTSTAYMELSSLRSEDTAVYFCARRIHYYDYFDYWGQGTLVTVSS

SEQ ID NO: 76 - protein, 112 aa, synthetic construct
  REGION 1..112: note = Description of the artificial sequence: DK1142 F21 and DK1142 F22 VL amino acid
DIVMTQSPLSLPVTLGEPASISCRSSQSIVHSNGNTYLEWYLQKPGQSPQLLIYKVSNRFSGVPDRFSGSGSGTDFTLKISRVEAEDVGVYYCFQGSHVPWTFGQGTKVEIK

SEQ ID NO: 77 - protein, 119 aa, synthetic construct
  REGION 1..119: note = Description of the artificial sequence: DK1142 F22 and DK1142 F24 VH amino acid
QVQLVQSGAELVKPGASVKVSCKASGYTFTSYNIHWVKQAPGQGLEWIGWIYPGDGNPKYNEKFKGKTTLTADKSTSTAYMELSSLRSEDTAVYFCARRIHYYDYFDYWGQGTLVTVSS

SEQ ID NO: 78 - protein, 112 aa, synthetic construct
  REGION 1..112: note = Description of the artificial sequence: DK1142 F24 VL amino acid
DVVMTQSPLSLPVTLGEPASISCRSSQSIVHSNGNTYLEWYLQKPGQSPKLLIYKISNRFSGVPDRFSGSGSGTDFTLKISRVEAEDVGVYYCFQGSHVPWTFGQGTKVEIK

SEQ ID NO: 79 - protein, 330 aa, Human [sequence omitted]

SEQ ID NO: 80 - protein, 330 aa, synthetic construct
  REGION 1..330: note = Description of the artificial sequence: IgG1 (S239C) amino acid
ASTKGPSVFPLAPSSKSTSGGTAALGCLVKDYFPEPVTVSWNSGALTSGVHTFPAVLQSSGLYSLSSVVTVPSSSLGTQTYICNVNHKPSNTKVDKKVEPKSCDKTHTCPPCPAPELLGGPCVFLFPPKPKDTLMISRTPEVTCVVVDVSHEDPEVKFNWYVDGVEVHNAKTKPREEQYNSTYRVVSVLTVLHQDWLNGKEYKCKVSNKALPAPIEKTISKAKGQPREPQVYTLPPSRDELTKNQVSLTCLVKGFYPSDIAVEWESNGQPENNYKTTPPVLDSDGSFFLYSKLTVDKSRWQQGNVFSCSVMHEALHNHYTQKSLSLSPGK